European Patent Application EP 4 198 142 A1, published June 21, 2023. Title: KIT AND METHOD FOR DETECTING NUCLEIC ACID AND USES THEREOF. Applicant: SHANGHAI EPIPROBE BIOTECHNOLOGY CO., LTD. The sequence listing filed with the application follows.

SEQUENCE LISTING (21 sequences)

SEQ ID NO: 1 - DNA, 58 bp, synthetic construct
cctacaacttgtgctaatgcactgccgcttccagttggtccagcatatgttttgtttc

SEQ ID NO: 2 - DNA, 33 bp, synthetic construct
gcttgatgagctttaccactgtctggcggtgac

SEQ ID NO: 3 - DNA, 35 bp, synthetic construct
tggcacgcaacgtcaatgaatatttcggtattcag

SEQ ID NO: 4 - DNA, 58 bp, synthetic construct
cctacaacttgtgctaatgcactgcagctcttacatacccttccactacggaggcagt

SEQ ID NO: 5 - DNA, 33 bp, synthetic construct
actgggttgatattcctcccgtggcttcaaagc

SEQ ID NO: 6 - DNA, 35 bp, synthetic construct
catcatcgcaccaggatcgtcaggggttttaatcg

SEQ ID NO: 7 - DNA, 57 bp, synthetic construct
cctacaacttgtgctaatgcactgggtgataactccttcactggccttgattgctga

SEQ ID NO: 8 - DNA, 33 bp, synthetic construct
agcggcttggttcgcctcccggcacgttcccac

SEQ ID NO: 9 - DNA, 35 bp, synthetic construct
cgctgtgggcaccagcagatcatccaggatcgatc

SEQ ID NO: 10 - DNA, 58 bp, synthetic construct
cctacaacttgtgctaatgcactgcaccgttatagcaacagccttcataggctacgtc

SEQ ID NO: 11 - DNA, 33 bp, synthetic construct
taagggatagctgatagtagatttgtgatgacc

SEQ ID NO: 12 - DNA, 35 bp, synthetic construct
gtagctcctcagaatgatatttgtcctcagggcag

SEQ ID NO: 13 - DNA, 59 bp, synthetic construct
cctacaacttgtgctaatgcactgcatatttcttcatgaagacctcacagtaaaaatag

SEQ ID NO: 14 - DNA, 34 bp, synthetic construct
ccacaaaatggatccagacaactgttcaaactga

SEQ ID NO: 15 - DNA, 31 bp, synthetic construct
gacccactccatcgagaagctagaccaaaat

SEQ ID NO: 16 - DNA, 60 bp, synthetic construct
cctacaacttgtgctaatgcactgcccccgccgggggcgcttcctcgccgctgccctccg

SEQ ID NO: 17 - DNA, 34 bp, synthetic construct
cctctccagcacgtccgcggccgcagcagccagc

SEQ ID NO: 18 - DNA, 33 bp, synthetic construct
agctgcgcgttgaccgcggggtccgacatgatg

SEQ ID NO: 19 - DNA, 30 bp, synthetic construct
cagccataacctttccacataccgcagacg

SEQ ID NO: 20 - DNA, 60 bp, synthetic construct
cctacaacttgtgctaatgcactgccctacaacttgtgctaatgaccctgtgggttttac

SEQ ID NO: 21 - DNA, 31 bp, synthetic construct
cccgtttaaaaacgattgtgcatcagctgac